European Patent Specification EP 3 010 517 B1, published April 8, 2026. Title: IMMUNOTHERAPY COMPOSITION AND USE THEREOF. Applicant: Ondek Pty Ltd. The sequence listing filed with the application follows.

SEQUENCE LISTING (4 sequences)

SEQ ID NO: 1 - DNA, 18 bp, artificial sequence
  Forward primer for H. pylori
ttggagggcttagtctct

SEQ ID NO: 2 - DNA, 20 bp, artificial sequence
  Reverse primer for H. pylori
aagattggctccacttcaca

SEQ ID NO: 3 - DNA, 10 bp, artificial sequence
  Primer 1254
ccgcagccaa

SEQ ID NO: 4 - DNA, 10 bp, artificial sequence
  Primer 1281
aacgcgcaac